European Patent Application EP 4 286 517 A2, published December 6, 2023. Title: Therapeutic Uses of Genome Editing With CRISPR/Cas Systems. Applicant: PRESIDENT AND FELLOWS OF HARVARD COLLEGE. Application EP. The sequence listing filed with the application follows.

SEQUENCE LISTING (353 sequences)

SEQ ID NO: 1 - DNA, 23 bp, synthetic construct
  misc_feature 1..23: note = CCR5 gRNA target site sequence
  source 1..23: mol_type = other DNA
tgacatcaattattatacatcgg

SEQ ID NO: 2 - DNA, 23 bp, synthetic construct
  misc_feature 1..23: note = CCR5 gRNA target site sequence
  source 1..23: mol_type = other DNA
cctgcctccgctctactcactgg

SEQ ID NO: 3 - DNA, 23 bp, synthetic construct
  misc_feature 1..23: note = CCR5 gRNA target site sequence
  source 1..23: mol_type = other DNA
tactcactggtgttcatctttgg

SEQ ID NO: 4 - DNA, 23 bp, synthetic construct
  misc_feature 1..23: note = CCR5 gRNA target site sequence
  source 1..23: mol_type = other DNA
ggtgttcatctttggttttgtgg

SEQ ID NO: 5 - DNA, 23 bp, synthetic construct
  misc_feature 1..23: note = CCR5 gRNA target site sequence
  source 1..23: mol_type = other DNA
gtgttcatctttggttttgtggg

SEQ ID NO: 6 - DNA, 23 bp, synthetic construct
  misc_feature 1..23: note = CCR5 gRNA target site sequence
  source 1..23: mol_type = other DNA
tggttttgtgggcaacatgctgg

SEQ ID NO: 7 - DNA, 23 bp, synthetic construct
  misc_feature 1..23: note = CCR5 gRNA target site sequence
  source 1..23: mol_type = other DNA
tcatcctgataaactgcaaaagg

SEQ ID NO: 8 - DNA, 23 bp, synthetic construct
  misc_feature 1..23: note = CCR5 gRNA target site sequence
  source 1..23: mol_type = other DNA
tgacatctacctgctcaacctgg

SEQ ID NO: 9 - DNA, 23 bp, synthetic construct
  misc_feature 1..23: note = CCR5 gRNA target site sequence
  source 1..23: mol_type = other DNA
tccttcttactgtccccttctgg

SEQ ID NO: 10 - DNA, 23 bp, synthetic construct
  misc_feature 1..23: note = CCR5 gRNA target site sequence
  source 1..23: mol_type = other DNA
ccttcttactgtccccttctggg

SEQ ID NO: 11 - DNA, 23 bp, synthetic construct
  misc_feature 1..23: note = CCR5 gRNA target site sequence
  source 1..23: mol_type = other DNA
ctcactatgctgccgcccagtgg

SEQ ID NO: 12 - DNA, 23 bp, synthetic construct
  misc_feature 1..23: note = CCR5 gRNA target site sequence
  source 1..23: mol_type = other DNA
tcactatgctgccgcccagtggg

SEQ ID NO: 13 - DNA, 23 bp, synthetic construct
  misc_feature 1..23: note = CCR5 gRNA target site sequence
  source 1..23: mol_type = other DNA
gctgccgcccagtgggactttgg

SEQ ID NO: 14 - DNA, 23 bp, synthetic construct
  misc_feature 1..23: note = CCR5 gRNA target site sequence
  source 1..23: mol_type = other DNA
acaatgtgtcaactcttgacagg

SEQ ID NO: 15 - DNA, 23 bp, synthetic construct
  misc_feature 1..23: note = CCR5 gRNA target site sequence
  source 1..23: mol_type = other DNA
caatgtgtcaactcttgacaggg

SEQ ID NO: 16 - DNA, 23 bp, synthetic construct
  misc_feature 1..23: note = CCR5 gRNA target site sequence
  source 1..23: mol_type = other DNA
ttgacagggctctattttatagg

SEQ ID NO: 17 - DNA, 23 bp, synthetic construct
  misc_feature 1..23: note = CCR5 gRNA target site sequence
  source 1..23: mol_type = other DNA
tattttataggcttcttctctgg

SEQ ID NO: 18 - DNA, 23 bp, synthetic construct
  misc_feature 1..23: note = CCR5 gRNA target site sequence
  source 1..23: mol_type = other DNA
tcatcctcctgacaatcgatagg

SEQ ID NO: 19 - DNA, 23 bp, synthetic construct
  misc_feature 1..23: note = CCR5 gRNA target site sequence
  source 1..23: mol_type = other DNA
cctgacaatcgataggtacctgg

SEQ ID NO: 20 - DNA, 23 bp, synthetic construct
  misc_feature 1..23: note = CCR5 gRNA target site sequence
  source 1..23: mol_type = other DNA
ctgtgtttgctttaaaagccagg

SEQ ID NO: 21 - DNA, 23 bp, synthetic construct
  misc_feature 1..23: note = CCR5 gRNA target site sequence
  source 1..23: mol_type = other DNA
gtttgctttaaaagccaggacgg

SEQ ID NO: 22 - DNA, 23 bp, synthetic construct
  misc_feature 1..23: note = CCR5 gRNA target site sequence
  source 1..23: mol_type = other DNA
aaagccaggacggtcacctttgg

SEQ ID NO: 23 - DNA, 23 bp, synthetic construct
  misc_feature 1..23: note = CCR5 gRNA target site sequence
  source 1..23: mol_type = other DNA
aagccaggacggtcacctttggg

SEQ ID NO: 24 - DNA, 23 bp, synthetic construct
  misc_feature 1..23: note = CCR5 gRNA target site sequence
  source 1..23: mol_type = other DNA
agccaggacggtcacctttgggg

SEQ ID NO: 25 - DNA, 23 bp, synthetic construct
  misc_feature 1..23: note = CCR5 gRNA target site sequence
  source 1..23: mol_type = other DNA
caggacggtcacctttggggtgg

SEQ ID NO: 26 - DNA, 23 bp, synthetic construct
  misc_feature 1..23: note = CCR5 gRNA target site sequence
  source 1..23: mol_type = other DNA
tggtgacaagtgtgatcacttgg

SEQ ID NO: 27 - DNA, 23 bp, synthetic construct
  misc_feature 1..23: note = CCR5 gRNA target site sequence
  source 1..23: mol_type = other DNA
ggtgacaagtgtgatcacttggg

SEQ ID NO: 28 - DNA, 23 bp, synthetic construct
  misc_feature 1..23: note = CCR5 gRNA target site sequence
  source 1..23: mol_type = other DNA
gacaagtgtgatcacttgggtgg

SEQ ID NO: 29 - DNA, 23 bp, synthetic construct
  misc_feature 1..23: note = CCR5 gRNA target site sequence
  source 1..23: mol_type = other DNA
aagtgtgatcacttgggtggtgg

SEQ ID NO: 30 - DNA, 23 bp, synthetic construct
  misc_feature 1..23: note = CCR5 gRNA target site sequence
  source 1..23: mol_type = other DNA
gctgtgtttgcgtctctcccagg

SEQ ID NO: 31 - DNA, 23 bp, synthetic construct
  misc_feature 1..23: note = CCR5 gRNA target site sequence
  source 1..23: mol_type = other DNA
tttaccagatctcaaaaagaagg

SEQ ID NO: 32 - DNA, 23 bp, synthetic construct
  misc_feature 1..23: note = CCR5 gRNA target site sequence
  source 1..23: mol_type = other DNA
catacagtcagtatcaattctgg

SEQ ID NO: 33 - DNA, 23 bp, synthetic construct
  misc_feature 1..23: note = CCR5 gRNA target site sequence
  source 1..23: mol_type = other DNA
gacattaaagatagtcatcttgg

SEQ ID NO: 34 - DNA, 23 bp, synthetic construct
  misc_feature 1..23: note = CCR5 gRNA target site sequence
  source 1..23: mol_type = other DNA
acattaaagatagtcatcttggg

SEQ ID NO: 35 - DNA, 23 bp, synthetic construct
  misc_feature 1..23: note = CCR5 gRNA target site sequence
  source 1..23: mol_type = other DNA
cattaaagatagtcatcttgggg

SEQ ID NO: 36 - DNA, 23 bp, synthetic construct
  misc_feature 1..23: note = CCR5 gRNA target site sequence
  source 1..23: mol_type = other DNA
aaagatagtcatcttggggctgg

SEQ ID NO: 37 - DNA, 23 bp, synthetic construct
  misc_feature 1..23: note = CCR5 gRNA target site sequence
  source 1..23: mol_type = other DNA
ggtcctgccgctgcttgtcatgg

SEQ ID NO: 38 - DNA, 23 bp, synthetic construct
  misc_feature 1..23: note = CCR5 gRNA target site sequence
  source 1..23: mol_type = other DNA
tgtcatggtcatctgctactcgg

SEQ ID NO: 39 - DNA, 23 bp, synthetic construct
  misc_feature 1..23: note = CCR5 gRNA target site sequence
  source 1..23: mol_type = other DNA
gtcatggtcatctgctactcggg

SEQ ID NO: 40 - DNA, 23 bp, synthetic construct
  misc_feature 1..23: note = CCR5 gRNA target site sequence
  source 1..23: mol_type = other DNA
gaatcctaaaaactctgcttcgg

SEQ ID NO: 41 - DNA, 23 bp, synthetic construct
  misc_feature 1..23: note = CCR5 gRNA target site sequence
  source 1..23: mol_type = other DNA
ggtgtcgaaatgagaagaagagg

SEQ ID NO: 42 - DNA, 23 bp, synthetic construct
  misc_feature 1..23: note = CCR5 gRNA target site sequence
  source 1..23: mol_type = other DNA
gaaatgagaagaagaggcacagg

SEQ ID NO: 43 - DNA, 23 bp, synthetic construct
  misc_feature 1..23: note = CCR5 gRNA target site sequence
  source 1..23: mol_type = other DNA
aaatgagaagaagaggcacaggg

SEQ ID NO: 44 - DNA, 23 bp, synthetic construct
  misc_feature 1..23: note = CCR5 gRNA target site sequence
  source 1..23: mol_type = other DNA
agaagaggcacagggctgtgagg

SEQ ID NO: 45 - DNA, 23 bp, synthetic construct
  misc_feature 1..23: note = CCR5 gRNA target site sequence
  source 1..23: mol_type = other DNA
tgattgtttattttctcttctgg

SEQ ID NO: 46 - DNA, 23 bp, synthetic construct
  misc_feature 1..23: note = CCR5 gRNA target site sequence
  source 1..23: mol_type = other DNA
gattgtttattttctcttctggg

SEQ ID NO: 47 - DNA, 23 bp, synthetic construct
  misc_feature 1..23: note = CCR5 gRNA target site sequence
  source 1..23: mol_type = other DNA
ccttctcctgaacaccttccagg

SEQ ID NO: 48 - DNA, 23 bp, synthetic construct
  misc_feature 1..23: note = CCR5 gRNA target site sequence
  source 1..23: mol_type = other DNA
aacaccttccaggaattctttgg

SEQ ID NO: 49 - DNA, 23 bp, synthetic construct
  misc_feature 1..23: note = CCR5 gRNA target site sequence
  source 1..23: mol_type = other DNA
ataattgcagtagctctaacagg

SEQ ID NO: 50 - DNA, 23 bp, synthetic construct
  misc_feature 1..23: note = CCR5 gRNA target site sequence
  source 1..23: mol_type = other DNA
ttgcagtagctctaacaggttgg

SEQ ID NO: 51 - DNA, 23 bp, synthetic construct
  misc_feature 1..23: note = CCR5 gRNA target site sequence
  source 1..23: mol_type = other DNA
caggttggaccaagctatgcagg

SEQ ID NO: 52 - DNA, 23 bp, synthetic construct
  misc_feature 1..23: note = CCR5 gRNA target site sequence
  source 1..23: mol_type = other DNA
atgcaggtgacagagactcttgg

SEQ ID NO: 53 - DNA, 23 bp, synthetic construct
  misc_feature 1..23: note = CCR5 gRNA target site sequence
  source 1..23: mol_type = other DNA
tgcaggtgacagagactcttggg

SEQ ID NO: 54 - DNA, 23 bp, synthetic construct
  misc_feature 1..23: note = CCR5 gRNA target site sequence
  source 1..23: mol_type = other DNA
cccatcatctatgcctttgtcgg

SEQ ID NO: 55 - DNA, 23 bp, synthetic construct
  misc_feature 1..23: note = CCR5 gRNA target site sequence
  source 1..23: mol_type = other DNA
ccatcatctatgcctttgtcggg

SEQ ID NO: 56 - DNA, 23 bp, synthetic construct
  misc_feature 1..23: note = CCR5 gRNA target site sequence
  source 1..23: mol_type = other DNA
catcatctatgcctttgtcgggg

SEQ ID NO: 57 - DNA, 23 bp, synthetic construct
  misc_feature 1..23: note = CCR5 gRNA target site sequence
  source 1..23: mol_type = other DNA
ctgttctattttccagcaagagg

SEQ ID NO: 58 - DNA, 23 bp, synthetic construct
  misc_feature 1..23: note = CCR5 gRNA target site sequence
  source 1..23: mol_type = other DNA
tcagtttacacccgatccactgg

SEQ ID NO: 59 - DNA, 23 bp, synthetic construct
  misc_feature 1..23: note = CCR5 gRNA target site sequence
  source 1..23: mol_type = other DNA
cagtttacacccgatccactggg

SEQ ID NO: 60 - DNA, 23 bp, synthetic construct
  misc_feature 1..23: note = CCR5 gRNA target site sequence
  source 1..23: mol_type = other DNA
agtttacacccgatccactgggg

SEQ ID NO: 61 - DNA, 23 bp, synthetic construct
  misc_feature 1..23: note = CCR5 gRNA target site sequence
  source 1..23: mol_type = other DNA
cacccgatccactggggagcagg

SEQ ID NO: 62 - DNA, 23 bp, synthetic construct
  misc_feature 1..23: note = CCR5 gRNA target site sequence
  source 1..23: mol_type = other DNA
tggggagcaggaaatatctgtgg

SEQ ID NO: 63 - DNA, 23 bp, synthetic construct
  misc_feature 1..23: note = CCR5 gRNA target site sequence
  source 1..23: mol_type = other DNA
ggggagcaggaaatatctgtggg

SEQ ID NO: 64 - DNA, 23 bp, synthetic construct
  misc_feature 1..23: note = CCR5 gRNA target site sequence
  source 1..23: mol_type = other DNA
taataattgatgtcatagattgg

SEQ ID NO: 65 - DNA, 23 bp, synthetic construct
  misc_feature 1..23: note = CCR5 gRNA target site sequence
  source 1..23: mol_type = other DNA
ttcacattgattttttggcaggg

SEQ ID NO: 66 - DNA, 23 bp, synthetic construct
  misc_feature 1..23: note = CCR5 gRNA target site sequence
  source 1..23: mol_type = other DNA
cttcacattgattttttggcagg

SEQ ID NO: 67 - DNA, 23 bp, synthetic construct
  misc_feature 1..23: note = CCR5 gRNA target site sequence
  source 1..23: mol_type = other DNA
tttgcttcacattgattttttgg

SEQ ID NO: 68 - DNA, 23 bp, synthetic construct
  misc_feature 1..23: note = CCR5 gRNA target site sequence
  source 1..23: mol_type = other DNA
gtagagcggaggcaggaggcggg

SEQ ID NO: 69 - DNA, 23 bp, synthetic construct
  misc_feature 1..23: note = CCR5 gRNA target site sequence
  source 1..23: mol_type = other DNA
agtagagcggaggcaggaggcgg

SEQ ID NO: 70 - DNA, 23 bp, synthetic construct
  misc_feature 1..23: note = CCR5 gRNA target site sequence
  source 1..23: mol_type = other DNA
gtgagtagagcggaggcaggagg

SEQ ID NO: 71 - DNA, 23 bp, synthetic construct
  misc_feature 1..23: note = CCR5 gRNA target site sequence
  source 1..23: mol_type = other DNA
ccagtgagtagagcggaggcagg

SEQ ID NO: 72 - DNA, 23 bp, synthetic construct
  misc_feature 1..23: note = CCR5 gRNA target site sequence
  source 1..23: mol_type = other DNA
aacaccagtgagtagagcggagg

SEQ ID NO: 73 - DNA, 23 bp, synthetic construct
  misc_feature 1..23: note = CCR5 gRNA target site sequence
  source 1..23: mol_type = other DNA
atgaacaccagtgagtagagcgg

SEQ ID NO: 74 - DNA, 23 bp, synthetic construct
  misc_feature 1..23: note = CCR5 gRNA target site sequence
  source 1..23: mol_type = other DNA
ttttgcagtttatcaggatgagg

SEQ ID NO: 75 - DNA, 23 bp, synthetic construct
  misc_feature 1..23: note = CCR5 gRNA target site sequence
  source 1..23: mol_type = other DNA
tcagccttttgcagtttatcagg

SEQ ID NO: 76 - DNA, 23 bp, synthetic construct
  misc_feature 1..23: note = CXCR5 gRNA target site sequence
  source 1..23: mol_type = other DNA
cagagatggccaggttgagcagg

SEQ ID NO: 77 - DNA, 23 bp, synthetic construct
  misc_feature 1..23: note = CCR5 gRNA target site sequence
  source 1..23: mol_type = other DNA
aaaacaggtcagagatggccagg

SEQ ID NO: 78 - DNA, 23 bp, synthetic construct
  misc_feature 1..23: note = CCR5 gRNA target site sequence
  source 1..23: mol_type = other DNA
aaggaaaaacaggtcagagatgg

SEQ ID NO: 79 - DNA, 23 bp, synthetic construct
  misc_feature 1..23: note = CCR5 gRNA target site sequence
  source 1..23: mol_type = other DNA
ggacagtaagaaggaaaaacagg

SEQ ID NO: 80 - DNA, 23 bp, synthetic construct
  misc_feature 1..23: note = CCR5 gRNA target site sequence
  source 1..23: mol_type = other DNA
cccagaaggggacagtaagaagg

SEQ ID NO: 81 - DNA, 23 bp, synthetic construct
  misc_feature 1..23: note = CCR5 gRNA target site sequence
  source 1..23: mol_type = other DNA
cagcatagtgagcccagaagggg

SEQ ID NO: 82 - DNA, 23 bp, synthetic construct
  misc_feature 1..23: note = CCR5 gRNA target site sequence
  source 1..23: mol_type = other DNA
gcagcatagtgagcccagaaggg

SEQ ID NO: 83 - DNA, 23 bp, synthetic construct
  misc_feature 1..23: note = CCR5 gRNA target site sequence
  source 1..23: mol_type = other DNA
ggcagcatagtgagcccagaagg

SEQ ID NO: 84 - DNA, 23 bp, synthetic construct
  misc_feature 1..23: note = CCR5 gRNA target site sequence
  source 1..23: mol_type = other DNA
atttccaaagtcccactgggcgg

SEQ ID NO: 85 - DNA, 23 bp, synthetic construct
  misc_feature 1..23: note = CCR5 gRNA target site sequence
  source 1..23: mol_type = other DNA
tgtatttccaaagtcccactggg

SEQ ID NO: 86 - DNA, 23 bp, synthetic construct
  misc_feature 1..23: note = CCR5 gRNA target site sequence
  source 1..23: mol_type = other DNA
ttgtatttccaaagtcccactgg

SEQ ID NO: 87 - DNA, 23 bp, synthetic construct
  misc_feature 1..23: note = CCR5 gRNA target site sequence
  source 1..23: mol_type = other DNA
ggtacctatcgattgtcaggagg

SEQ ID NO: 88 - DNA, 23 bp, synthetic construct
  misc_feature 1..23: note = CCR5 gRNA target site sequence
  source 1..23: mol_type = other DNA
ccaggtacctatcgattgtcagg

SEQ ID NO: 89 - DNA, 23 bp, synthetic construct
  misc_feature 1..23: note = CCR5 gRNA target site sequence
  source 1..23: mol_type = other DNA
acacagcatggacgacagccagg

SEQ ID NO: 90 - DNA, 23 bp, synthetic construct
  misc_feature 1..23: note = CCR5 gRNA target site sequence
  source 1..23: mol_type = other DNA
cttttaaagcaaacacagcatgg

SEQ ID NO: 91 - DNA, 23 bp, synthetic construct
  misc_feature 1..23: note = CCR5 gRNA target site sequence
  source 1..23: mol_type = other DNA
caccccaaaggtgaccgtcctgg

SEQ ID NO: 92 - DNA, 23 bp, synthetic construct
  misc_feature 1..23: note = CCR5 gRNA target site sequence
  source 1..23: mol_type = other DNA
cacacttgtcaccaccccaaagg

SEQ ID NO: 93 - DNA, 23 bp, synthetic construct
  misc_feature 1..23: note = CCR5 gRNA target site sequence
  source 1..23: mol_type = other DNA
atctggtaaagatgattcctggg

SEQ ID NO: 94 - DNA, 23 bp, synthetic construct
  misc_feature 1..23: note = CCR5 gRNA target site sequence
  source 1..23: mol_type = other DNA
gatctggtaaagatgattcctgg

SEQ ID NO: 95 - DNA, 23 bp, synthetic construct
  misc_feature 1..23: note = CCR5 gRNA target site sequence
  source 1..23: mol_type = other DNA
aagaccttctttttgagatctgg

SEQ ID NO: 96 - DNA, 23 bp, synthetic construct
  misc_feature 1..23: note = CCR5 gRNA target site sequence
  source 1..23: mol_type = other DNA
gtatggaaaatgagagctgcagg

SEQ ID NO: 97 - DNA, 23 bp, synthetic construct
  misc_feature 1..23: note = CCR5 gRNA target site sequence
  source 1..23: mol_type = other DNA
cagaattgatactgactgtatgg

SEQ ID NO: 98 - DNA, 23 bp, synthetic construct
  misc_feature 1..23: note = CCR5 gRNA target site sequence
  source 1..23: mol_type = other DNA
agatgactatctttaatgtctgg

SEQ ID NO: 99 - DNA, 23 bp, synthetic construct
  misc_feature 1..23: note = CCR5 gRNA target site sequence
  source 1..23: mol_type = other DNA
tgaccatgacaagcagcggcagg

SEQ ID NO: 100 - DNA, 23 bp, synthetic construct
  misc_feature 1..23: note = CCR5 gRNA target site sequence
  source 1..23: mol_type = other DNA
cagatgaccatgacaagcagcgg

SEQ ID NO: 101 - DNA, 23 bp, synthetic construct
  misc_feature 1..23: note = CCR5 gRNA target site sequence
  source 1..23: mol_type = other DNA
gacaccgaagcagagtttttagg

SEQ ID NO: 102 - DNA, 23 bp, synthetic construct
  misc_feature 1..23: note = CCR5 gRNA target site sequence
  source 1..23: mol_type = other DNA
gagaaaataaacaatcatgatgg

SEQ ID NO: 103 - DNA, 23 bp, synthetic construct
  misc_feature 1..23: note = CCR5 gRNA target site sequence
  source 1..23: mol_type = other DNA
aggagaaggacaatgttgtaggg

SEQ ID NO: 104 - DNA, 23 bp, synthetic construct
  misc_feature 1..23: note = CCR5 gRNA target site sequence
  source 1..23: mol_type = other DNA
caggagaaggacaatgttgtagg

SEQ ID NO: 105 - DNA, 23 bp, synthetic construct
  misc_feature 1..23: note = CCR5 gRNA target site sequence
  source 1..23: mol_type = other DNA
cctggaaggtgttcaggagaagg

SEQ ID NO: 106 - DNA, 23 bp, synthetic construct
  misc_feature 1..23: note = CCR5 gRNA target site sequence
  source 1..23: mol_type = other DNA
agaattcctggaaggtgttcagg

SEQ ID NO: 107 - DNA, 23 bp, synthetic construct
  misc_feature 1..23: note = CCR5 gRNA target site sequence
  source 1..23: mol_type = other DNA
caggccaaagaattcctggaagg

SEQ ID NO: 108 - DNA, 23 bp, synthetic construct
  misc_feature 1..23: note = CCR5 gRNA target site sequence
  source 1..23: mol_type = other DNA
tattcaggccaaagaattcctgg

SEQ ID NO: 109 - DNA, 23 bp, synthetic construct
  misc_feature 1..23: note = CCR5 gRNA target site sequence
  source 1..23: mol_type = other DNA
tagagctactgcaattattcagg

SEQ ID NO: 110 - DNA, 23 bp, synthetic construct
  misc_feature 1..23: note = CCR5 gRNA target site sequence
  source 1..23: mol_type = other DNA
tctctgtcacctgcatagcttgg

SEQ ID NO: 111 - DNA, 23 bp, synthetic construct
  misc_feature 1..23: note = CCR5 gRNA target site sequence
  source 1..23: mol_type = other DNA
cgacaaaggcatagatgatgggg

SEQ ID NO: 112 - DNA, 23 bp, synthetic construct
  misc_feature 1..23: note = CCR5 gRNA target site sequence
  source 1..23: mol_type = other DNA
ccgacaaaggcatagatgatggg

SEQ ID NO: 113 - DNA, 23 bp, synthetic construct
  misc_feature 1..23: note = CCR5 gRNA target site sequence
  source 1..23: mol_type = other DNA
cccgacaaaggcatagatgatgg

SEQ ID NO: 114 - DNA, 23 bp, synthetic construct
  misc_feature 1..23: note = CCR5 gRNA target site sequence
  source 1..23: mol_type = other DNA
tctgaacttctccccgacaaagg

SEQ ID NO: 115 - DNA, 23 bp, synthetic construct
  misc_feature 1..23: note = CCR5 gRNA target site sequence
  source 1..23: mol_type = other DNA
gcttttggaagaagactaagagg

SEQ ID NO: 116 - DNA, 23 bp, synthetic construct
  misc_feature 1..23: note = CCR5 gRNA target site sequence
  source 1..23: mol_type = other DNA
agcgtttggcaatgtgcttttgg

SEQ ID NO: 117 - DNA, 23 bp, synthetic construct
  misc_feature 1..23: note = CCR5 gRNA target site sequence
  source 1..23: mol_type = other DNA
acagcatttgcagaagcgtttgg

SEQ ID NO: 118 - DNA, 23 bp, synthetic construct
  misc_feature 1..23: note = CCR5 gRNA target site sequence
  source 1..23: mol_type = other DNA
ctcgctcgggagcctcttgctgg

SEQ ID NO: 119 - DNA, 23 bp, synthetic construct
  misc_feature 1..23: note = CCR5 gRNA target site sequence
  source 1..23: mol_type = other DNA
taaactgagcttgctcgctcggg

SEQ ID NO: 120 - DNA, 23 bp, synthetic construct
  misc_feature 1..23: note = CCR5 gRNA target site sequence
  source 1..23: mol_type = other DNA
gtaaactgagcttgctcgctcgg

SEQ ID NO: 121 - DNA, 23 bp, synthetic construct
  misc_feature 1..23: note = CCR5 gRNA target site sequence
  source 1..23: mol_type = other DNA
ttcctgctccccagtggatcggg

SEQ ID NO: 122 - DNA, 23 bp, synthetic construct
  misc_feature 1..23: note = CCR5 gRNA target site sequence
  source 1..23: mol_type = other DNA
tttcctgctccccagtggatcgg

SEQ ID NO: 123 - DNA, 23 bp, synthetic construct
  misc_feature 1..23: note = CCR5 gRNA target site sequence
  source 1..23: mol_type = other DNA
agatatttcctgctccccagtgg

SEQ ID NO: 124 - DNA, 28 bp, synthetic construct
  misc_feature 1..28: note = CCR5 gRNA target site sequence
  source 1..28: mol_type = other DNA
atcatctttaccagatctcaaaaagaag

SEQ ID NO: 125 - DNA, 28 bp, synthetic construct
  misc_feature 1..28: note = CCR5 gRNA target site sequence
  source 1..28: mol_type = other DNA
aactctgcttcggtgtcgaaatgagaag

SEQ ID NO: 126 - DNA, 28 bp, synthetic construct
  misc_feature 1..28: note = CCR5 gRNA target site sequence
  source 1..28: mol_type = other DNA
tctgcttcggtgtcgaaatgagaagaag

SEQ ID NO: 127 - DNA, 28 bp, synthetic construct
  misc_feature 1..28: note = CCR5 gRNA target site sequence
  source 1..28: mol_type = other DNA
catcatctatgcctttgtcggggagaag

SEQ ID NO: 128 - DNA, 28 bp, synthetic construct
  misc_feature 1..28: note = CCR5 gRNA target site sequence
  source 1..28: mol_type = other DNA
atgcctttgtcggggagaagttcagaaa

SEQ ID NO: 129 - DNA, 28 bp, synthetic construct
  misc_feature 1..28: note = CCR5 gRNA target site sequence
  source 1..28: mol_type = other DNA
agtgagcccagaaggggacagtaagaag

SEQ ID NO: 130 - DNA, 28 bp, synthetic construct
  misc_feature 1..28: note = CCR5 gRNA target site sequence
  source 1..28: mol_type = other DNA
ctgggcggcagcatagtgagcccagaag

SEQ ID NO: 131 - DNA, 28 bp, synthetic construct
  misc_feature 1..28: note = CCR5 gRNA target site sequence
  source 1..28: mol_type = other DNA
gatgatgaagaagattccagagaagaag

SEQ ID NO: 132 - DNA, 28 bp, synthetic construct
  misc_feature 1..28: note = CCR5 gRNA target site sequence
  source 1..28: mol_type = other DNA
gaggatgatgaagaagattccagagaag

SEQ ID NO: 133 - DNA, 28 bp, synthetic construct
  misc_feature 1..28: note = CCR5 gRNA target site sequence
  source 1..28: mol_type = other DNA
atcgattgtcaggaggatgatgaagaag

SEQ ID NO: 134 - DNA, 28 bp, synthetic construct
  misc_feature 1..28: note = CCR5 gRNA target site sequence
  source 1..28: mol_type = other DNA
caatgttgtagggagcccagaagagaaa

SEQ ID NO: 135 - DNA, 28 bp, synthetic construct
  misc_feature 1..28: note = CCR5 gRNA target site sequence
  source 1..28: mol_type = other DNA
aaggacaatgttgtagggagcccagaag

SEQ ID NO: 136 - DNA, 28 bp, synthetic construct
  misc_feature 1..28: note = CCR5 gRNA target site sequence
  source 1..28: mol_type = other DNA
agaattcctggaaggtgttcaggagaag

SEQ ID NO: 137 - DNA, 28 bp, synthetic construct
  misc_feature 1..28: note = CCR5 gRNA target site sequence
  source 1..28: mol_type = other DNA
gcgtttggcaatgtgcttttggaagaag

SEQ ID NO: 138 - DNA, 28 bp, synthetic construct
  misc_feature 1..28: note = CCR5 gRNA target site sequence
  source 1..28: mol_type = other DNA
ctggaaaatagaacagcatttgcagaag

SEQ ID NO: 139 - DNA, 28 bp, synthetic construct
  misc_feature 1..28: note = CCR5 gRNA target site sequence
  source 1..28: mol_type = other DNA
tcgggagcctcttgctggaaaatagaac

SEQ ID NO: 140 - DNA, 23 bp, synthetic construct
  misc_feature 1..23: note = CXCR4 gRNA target site sequence
  source 1..23: mol_type = other DNA
acttgaagactcagactcagtgg

SEQ ID NO: 141 - DNA, 23 bp, synthetic construct
  misc_feature 1..23: note = CXCR4 gRNA target site sequence
  source 1..23: mol_type = other DNA
atgtccacctcgctttcctttgg

SEQ ID NO: 142 - DNA, 23 bp, synthetic construct
  misc_feature 1..23: note = CXCR4 gRNA target site sequence
  source 1..23: mol_type = other DNA
cacctcgctttcctttggagagg

SEQ ID NO: 143 - DNA, 23 bp, synthetic construct
  misc_feature 1..23: note = CXCR4 gRNA target site sequence
  source 1..23: mol_type = other DNA
ttcctttggagaggatcttgagg

SEQ ID NO: 144 - DNA, 23 bp, synthetic construct
  misc_feature 1..23: note = CXCR4 gRNA target site sequence
  source 1..23: mol_type = other DNA
tttggagaggatcttgaggctgg

SEQ ID NO: 145 - DNA, 23 bp, synthetic construct
  misc_feature 1..23: note = CXCR4 gRNA target site sequence
  source 1..23: mol_type = other DNA
gctggaccctctgctcacagagg

SEQ ID NO: 146 - DNA, 23 bp, synthetic construct
  misc_feature 1..23: note = CXCR4 gRNA target site sequence
  source 1..23: mol_type = other DNA
tcacagaggtgagtgcgtgctgg

SEQ ID NO: 147 - DNA, 23 bp, synthetic construct
  misc_feature 1..23: note = CXCR4 gRNA target site sequence
  source 1..23: mol_type = other DNA
cacagaggtgagtgcgtgctggg

SEQ ID NO: 148 - DNA, 23 bp, synthetic construct
  misc_feature 1..23: note = CXCR4 gRNA target site sequence
  source 1..23: mol_type = other DNA
ggtgagtgcgtgctgggcagagg

SEQ ID NO: 149 - DNA, 23 bp, synthetic construct
  misc_feature 1..23: note = CXCR4 gRNA target site sequence
  source 1..23: mol_type = other DNA
ctgggcagaggttttaaatttgg

SEQ ID NO: 150 - DNA, 23 bp, synthetic construct
  misc_feature 1..23: note = CXCR4 gRNA target site sequence
  source 1..23: mol_type = other DNA
aggttttaaatttggctccaagg

SEQ ID NO: 151 - DNA, 23 bp, synthetic construct
  misc_feature 1..23: note = CXCR4 gRNA target site sequence
  source 1..23: mol_type = other DNA
tggctccaaggaaagcatagagg

SEQ ID NO: 152 - DNA, 23 bp, synthetic construct
  misc_feature 1..23: note = CXCR4 gRNA target site sequence
  source 1..23: mol_type = other DNA
tccaaggaaagcatagaggatgg

SEQ ID NO: 153 - DNA, 23 bp, synthetic construct
  misc_feature 1..23: note = CXCR4 gRNA target site sequence
  source 1..23: mol_type = other DNA
ccaaggaaagcatagaggatggg

SEQ ID NO: 154 - DNA, 23 bp, synthetic construct
  misc_feature 1..23: note = CXCR4 gRNA target site sequence
  source 1..23: mol_type = other DNA
caaggaaagcatagaggatgggg

SEQ ID NO: 155 - DNA, 23 bp, synthetic construct
  misc_feature 1..23: note = CXCR4 gRNA target site sequence
  source 1..23: mol_type = other DNA
ggatggggttcagacaacagtgg

SEQ ID NO: 156 - DNA, 23 bp, synthetic construct
  misc_feature 1..23: note = CXCR4 gRNA target site sequence
  source 1..23: mol_type = other DNA
gacaacagtggaagaaagctagg

SEQ ID NO: 157 - DNA, 23 bp, synthetic construct
  misc_feature 1..23: note = CXCR4 gRNA target site sequence
  source 1..23: mol_type = other DNA
acaacagtggaagaaagctaggg

SEQ ID NO: 158 - DNA, 23 bp, synthetic construct
  misc_feature 1..23: note = CXCR4 gRNA target site sequence
  source 1..23: mol_type = other DNA
gtggaagaaagctagggcctcgg

SEQ ID NO: 159 - DNA, 23 bp, synthetic construct
  misc_feature 1..23: note = CXCR4 gRNA target site sequence
  source 1..23: mol_type = other DNA
gaaagctagggcctcggtgatgg

SEQ ID NO: 160 - DNA, 23 bp, synthetic construct
  misc_feature 1..23: note = CXCR4 gRNA target site sequence
  source 1..23: mol_type = other DNA
acccttgcttgatgatttccagg

SEQ ID NO: 161 - DNA, 23 bp, synthetic construct
  misc_feature 1..23: note = CXCR4 gRNA target site sequence
  source 1..23: mol_type = other DNA
cttgcttgatgatttccaggagg

SEQ ID NO: 162 - DNA, 23 bp, synthetic construct
  misc_feature 1..23: note = CXCR4 gRNA target site sequence
  source 1..23: mol_type = other DNA
gatgatttccaggaggatgaagg

SEQ ID NO: 163 - DNA, 23 bp, synthetic construct
  misc_feature 1..23: note = CXCR4 gRNA target site sequence
  source 1..23: mol_type = other DNA
atgctgatcccaatgtagtaagg

SEQ ID NO: 164 - DNA, 23 bp, synthetic construct
  misc_feature 1..23: note = CXCR4 gRNA target site sequence
  source 1..23: mol_type = other DNA
aatgtagtaaggcagccaacagg

SEQ ID NO: 165 - DNA, 23 bp, synthetic construct
  misc_feature 1..23: note = CXCR4 gRNA target site sequence
  source 1..23: mol_type = other DNA
gccaacaggcgaagaaagccagg

SEQ ID NO: 166 - DNA, 23 bp, synthetic construct
  misc_feature 1..23: note = CXCR4 gRNA target site sequence
  source 1..23: mol_type = other DNA
aggcgaagaaagccaggatgagg

SEQ ID NO: 167 - DNA, 23 bp, synthetic construct
  misc_feature 1..23: note = CXCR4 gRNA target site sequence
  source 1..23: mol_type = other DNA
agccaggatgaggatgactgtgg

SEQ ID NO: 168 - DNA, 23 bp, synthetic construct
  misc_feature 1..23: note = CXCR4 gRNA target site sequence
  source 1..23: mol_type = other DNA
tgaggatgactgtggtcttgagg

SEQ ID NO: 169 - DNA, 23 bp, synthetic construct
  misc_feature 1..23: note = CXCR4 gRNA target site sequence
  source 1..23: mol_type = other DNA
gaggatgactgtggtcttgaggg

SEQ ID NO: 170 - DNA, 23 bp, synthetic construct
  misc_feature 1..23: note = CXCR4 gRNA target site sequence
  source 1..23: mol_type = other DNA
tcttgagggccttgcgcttctgg

SEQ ID NO: 171 - DNA, 23 bp, synthetic construct
  misc_feature 1..23: note = CXCR4 gRNA target site sequence
  source 1..23: mol_type = other DNA
tgagggccttgcgcttctggtgg

SEQ ID NO: 172 - DNA, 23 bp, synthetic construct
  misc_feature 1..23: note = CXCR4 gRNA target site sequence
  source 1..23: mol_type = other DNA
cttgcgcttctggtggcccttgg

SEQ ID NO: 173 - DNA, 23 bp, synthetic construct
  misc_feature 1..23: note = CXCR4 gRNA target site sequence
  source 1..23: mol_type = other DNA
gcccttggagtgtgacagcttgg

SEQ ID NO: 174 - DNA, 23 bp, synthetic construct
  misc_feature 1..23: note = CXCR4 gRNA target site sequence
  source 1..23: mol_type = other DNA
ggagatgataatgcaatagcagg

SEQ ID NO: 175 - DNA, 23 bp, synthetic construct
  misc_feature 1..23: note = CXCR4 gRNA target site sequence
  source 1..23: mol_type = other DNA
tgataatgcaatagcaggacagg

SEQ ID NO: 176 - DNA, 23 bp, synthetic construct
  misc_feature 1..23: note = CXCR4 gRNA target site sequence
  source 1..23: mol_type = other DNA
caggacaggatgacaataccagg

SEQ ID NO: 177 - DNA, 23 bp, synthetic construct
  misc_feature 1..23: note = CXCR4 gRNA target site sequence
  source 1..23: mol_type = other DNA
acaggatgacaataccaggcagg

SEQ ID NO: 178 - DNA, 23 bp, synthetic construct
  misc_feature 1..23: note = CXCR4 gRNA target site sequence
  source 1..23: mol_type = other DNA
tgacaataccaggcaggataagg

SEQ ID NO: 179 - DNA, 23 bp, synthetic construct
  misc_feature 1..23: note = CXCR4 gRNA target site sequence
  source 1..23: mol_type = other DNA
caaccatgatgtgctgaaactgg

SEQ ID NO: 180 - DNA, 23 bp, synthetic construct
  misc_feature 1..23: note = CXCR4 gRNA target site sequence
  source 1..23: mol_type = other DNA
cacaaccacccacaagtcattgg

SEQ ID NO: 181 - DNA, 23 bp, synthetic construct
  misc_feature 1..23: note = CXCR4 gRNA target site sequence
  source 1..23: mol_type = other DNA
acaaccacccacaagtcattggg

SEQ ID NO: 182 - DNA, 23 bp, synthetic construct
  misc_feature 1..23: note = CXCR4 gRNA target site sequence
  source 1..23: mol_type = other DNA
caaccacccacaagtcattgggg

SEQ ID NO: 183 - DNA, 23 bp, synthetic construct
  misc_feature 1..23: note = CXCR4 gRNA target site sequence
  source 1..23: mol_type = other DNA
acaagtcattggggtagaagcgg

SEQ ID NO: 184 - DNA, 23 bp, synthetic construct
  misc_feature 1..23: note = CXCR4 gRNA target site sequence
  source 1..23: mol_type = other DNA
gtcatctgcctcactgacgttgg

SEQ ID NO: 185 - DNA, 23 bp, synthetic construct
  misc_feature 1..23: note = CXCR4 gRNA target site sequence
  source 1..23: mol_type = other DNA
gacgttggcaaagatgaagtcgg

SEQ ID NO: 186 - DNA, 23 bp, synthetic construct
  misc_feature 1..23: note = CXCR4 gRNA target site sequence
  source 1..23: mol_type = other DNA
acgttggcaaagatgaagtcggg

SEQ ID NO: 187 - DNA, 23 bp, synthetic construct
  misc_feature 1..23: note = CXCR4 gRNA target site sequence
  source 1..23: mol_type = other DNA
tgaagtcgggaatagtcagcagg

SEQ ID NO: 188 - DNA, 23 bp, synthetic construct
  misc_feature 1..23: note = CXCR4 gRNA target site sequence
  source 1..23: mol_type = other DNA
agtcgggaatagtcagcaggagg

SEQ ID NO: 189 - DNA, 23 bp, synthetic construct
  misc_feature 1..23: note = CXCR4 gRNA target site sequence
  source 1..23: mol_type = other DNA
gtcgggaatagtcagcaggaggg

SEQ ID NO: 190 - DNA, 23 bp, synthetic construct
  misc_feature 1..23: note = CXCR4 gRNA target site sequence
  source 1..23: mol_type = other DNA
ggaatagtcagcaggagggcagg

SEQ ID NO: 191 - DNA, 23 bp, synthetic construct
  misc_feature 1..23: note = CXCR4 gRNA target site sequence
  source 1..23: mol_type = other DNA
gaatagtcagcaggagggcaggg

SEQ ID NO: 192 - DNA, 23 bp, synthetic construct
  misc_feature 1..23: note = CXCR4 gRNA target site sequence
  source 1..23: mol_type = other DNA
ttttcagccaacagcttccttgg

SEQ ID NO: 193 - DNA, 23 bp, synthetic construct
  misc_feature 1..23: note = CXCR4 gRNA target site sequence
  source 1..23: mol_type = other DNA
cttccttggcctctgactgttgg

SEQ ID NO: 194 - DNA, 23 bp, synthetic construct
  misc_feature 1..23: note = CXCR4 gRNA target site sequence
  source 1..23: mol_type = other DNA
ccttggcctctgactgttggtgg

SEQ ID NO: 195 - DNA, 23 bp, synthetic construct
  misc_feature 1..23: note = CXCR4 gRNA target site sequence
  source 1..23: mol_type = other DNA
gcctctgactgttggtggcgtgg

SEQ ID NO: 196 - DNA, 23 bp, synthetic construct
  misc_feature 1..23: note = CXCR4 gRNA target site sequence
  source 1..23: mol_type = other DNA
actgttggtggcgtggacgatgg

SEQ ID NO: 197 - DNA, 23 bp, synthetic construct
  misc_feature 1..23: note = CXCR4 gRNA target site sequence
  source 1..23: mol_type = other DNA
tggtggcgtggacgatggccagg

SEQ ID NO: 198 - DNA, 23 bp, synthetic construct
  misc_feature 1..23: note = CXCR4 gRNA target site sequence
  source 1..23: mol_type = other DNA
cgtggacgatggccaggtagcgg

SEQ ID NO: 199 - DNA, 23 bp, synthetic construct
  misc_feature 1..23: note = CXCR4 gRNA target site sequence
  source 1..23: mol_type = other DNA
gtagcggtccagactgatgaagg

SEQ ID NO: 200 - DNA, 23 bp, synthetic construct
  misc_feature 1..23: note = CXCR4 gRNA target site sequence
  source 1..23: mol_type = other DNA
ggtccagactgatgaaggccagg

SEQ ID NO: 201 - DNA, 23 bp, synthetic construct
  misc_feature 1..23: note = CXCR4 gRNA target site sequence
  source 1..23: mol_type = other DNA
gactgatgaaggccaggatgagg

SEQ ID NO: 202 - DNA, 23 bp, synthetic construct
  misc_feature 1..23: note = CXCR4 gRNA target site sequence
  source 1..23: mol_type = other DNA
ggatgaggacactgctgtagagg

SEQ ID NO: 203 - DNA, 23 bp, synthetic construct
  misc_feature 1..23: note = CXCR4 gRNA target site sequence
  source 1..23: mol_type = other DNA
ggttgactgtgtagatgacatgg

SEQ ID NO: 204 - DNA, 23 bp, synthetic construct
  misc_feature 1..23: note = CXCR4 gRNA target site sequence
  source 1..23: mol_type = other DNA
tgacatggactgccttgcatagg

SEQ ID NO: 205 - DNA, 23 bp, synthetic construct
  misc_feature 1..23: note = CXCR4 gRNA target site sequence
  source 1..23: mol_type = other DNA
cccaaagtaccagtttgccacgg

SEQ ID NO: 206 - DNA, 23 bp, synthetic construct
  misc_feature 1..23: note = CXCR4 gRNA target site sequence
  source 1..23: mol_type = other DNA
cacggcatcaactgcccagaagg

SEQ ID NO: 207 - DNA, 23 bp, synthetic construct
  misc_feature 1..23: note = CXCR4 gRNA target site sequence
  source 1..23: mol_type = other DNA
acggcatcaactgcccagaaggg

SEQ ID NO: 208 - DNA, 23 bp, synthetic construct
  misc_feature 1..23: note = CXCR4 gRNA target site sequence
  source 1..23: mol_type = other DNA
agggaagcgtgatgacaaagagg

SEQ ID NO: 209 - DNA, 23 bp, synthetic construct
  misc_feature 1..23: note = CXCR4 gRNA target site sequence
  source 1..23: mol_type = other DNA
gaagcgtgatgacaaagaggagg

SEQ ID NO: 210 - DNA, 23 bp, synthetic construct
  misc_feature 1..23: note = CXCR4 gRNA target site sequence
  source 1..23: mol_type = other DNA
cgtgatgacaaagaggaggtcgg

SEQ ID NO: 211 - DNA, 23 bp, synthetic construct
  misc_feature 1..23: note = CXCR4 gRNA target site sequence
  source 1..23: mol_type = other DNA
agaggaggtcggccactgacagg

SEQ ID NO: 212 - DNA, 23 bp, synthetic construct
  misc_feature 1..23: note = CXCR4 gRNA target site sequence
  source 1..23: mol_type = other DNA
tcatgcttctcagtttcttctgg

SEQ ID NO: 213 - DNA, 23 bp, synthetic construct
  misc_feature 1..23: note = CXCR4 gRNA target site sequence
  source 1..23: mol_type = other DNA
tcttctggtaacccatgaccagg

SEQ ID NO: 214 - DNA, 23 bp, synthetic construct
  misc_feature 1..23: note = CXCR4 gRNA target site sequence
  source 1..23: mol_type = other DNA
aatgccagttaagaagatgatgg

SEQ ID NO: 215 - DNA, 23 bp, synthetic construct
  misc_feature 1..23: note = CXCR4 gRNA target site sequence
  source 1..23: mol_type = other DNA
taagaagatgatggagtagatgg

SEQ ID NO: 216 - DNA, 23 bp, synthetic construct
  misc_feature 1..23: note = CXCR4 gRNA target site sequence
  source 1..23: mol_type = other DNA
gaagatgatggagtagatggtgg

SEQ ID NO: 217 - DNA, 23 bp, synthetic construct
  misc_feature 1..23: note = CXCR4 gRNA target site sequence
  source 1..23: mol_type = other DNA
aagatgatggagtagatggtggg

SEQ ID NO: 218 - DNA, 23 bp, synthetic construct
  misc_feature 1..23: note = CXCR4 gRNA target site sequence
  source 1..23: mol_type = other DNA
tgatggagtagatggtgggcagg

SEQ ID NO: 219 - DNA, 23 bp, synthetic construct
  misc_feature 1..23: note = CXCR4 gRNA target site sequence
  source 1..23: mol_type = other DNA
tgaaattagcattttcttcacgg

SEQ ID NO: 220 - DNA, 23 bp, synthetic construct
  misc_feature 1..23: note = CXCR4 gRNA target site sequence
  source 1..23: mol_type = other DNA
agcattttcttcacggaaacagg

SEQ ID NO: 221 - DNA, 23 bp, synthetic construct
  misc_feature 1..23: note = CXCR4 gRNA target site sequence
  source 1..23: mol_type = other DNA
gcattttcttcacggaaacaggg

SEQ ID NO: 222 - DNA, 23 bp, synthetic construct
  misc_feature 1..23: note = CXCR4 gRNA target site sequence
  source 1..23: mol_type = other DNA
acggaaacagggttccttcatgg

SEQ ID NO: 223 - DNA, 23 bp, synthetic construct
  misc_feature 1..23: note = CXCR4 gRNA target site sequence
  source 1..23: mol_type = other DNA
gtcccctgagcccatttcctcgg

SEQ ID NO: 224 - DNA, 23 bp, synthetic construct
  misc_feature 1..23: note = CXCR4 gRNA target site sequence
  source 1..23: mol_type = other DNA
gaagtgtatatctgcaaaagagg

SEQ ID NO: 225 - DNA, 23 bp, synthetic construct
  misc_feature 1..23: note = CXCR4 gRNA target site sequence
  source 1..23: mol_type = other DNA
tatatctgcaaaagaggcaaagg

SEQ ID NO: 226 - DNA, 23 bp, synthetic construct
  misc_feature 1..23: note = CXCR4 gRNA target site sequence
  source 1..23: mol_type = other DNA
ctgcaaaagaggcaaaggaatgg

SEQ ID NO: 227 - DNA, 23 bp, synthetic construct
  misc_feature 1..23: note = CXCR4 gRNA target site sequence
  source 1..23: mol_type = other DNA
ctctccaaaggaaagcgaggtgg

SEQ ID NO: 228 - DNA, 23 bp, synthetic construct
  misc_feature 1..23: note = CXCR4 gRNA target site sequence
  source 1..23: mol_type = other DNA
atcctctccaaaggaaagcgagg

SEQ ID NO: 229 - DNA, 23 bp, synthetic construct
  misc_feature 1..23: note = CXCR4 gRNA target site sequence
  source 1..23: mol_type = other DNA
agcctcaagatcctctccaaagg

SEQ ID NO: 230 - DNA, 23 bp, synthetic construct
  misc_feature 1..23: note = CXCR4 gRNA target site sequence
  source 1..23: mol_type = other DNA
cactcacctctgtgagcagaggg

SEQ ID NO: 231 - DNA, 23 bp, synthetic construct
  misc_feature 1..23: note = CXCR4 gRNA target site sequence
  source 1..23: mol_type = other DNA
gcactcacctctgtgagcagagg

SEQ ID NO: 232 - DNA, 23 bp, synthetic construct
  misc_feature 1..23: note = CXCR4 gRNA target site sequence
  source 1..23: mol_type = other DNA
cccatcctctatgctttccttgg

SEQ ID NO: 233 - DNA, 23 bp, synthetic construct
  misc_feature 1..23: note = CXCR4 gRNA target site sequence
  source 1..23: mol_type = other DNA
caagtggatttccatcaccgagg

SEQ ID NO: 234 - DNA, 23 bp, synthetic construct
  misc_feature 1..23: note = CXCR4 gRNA target site sequence
  source 1..23: mol_type = other DNA
ttgagaacactgtgcacaagtgg

SEQ ID NO: 235 - DNA, 23 bp, synthetic construct
  misc_feature 1..23: note = CXCR4 gRNA target site sequence
  source 1..23: mol_type = other DNA
tcctggaaatcatcaagcaaggg

SEQ ID NO: 236 - DNA, 23 bp, synthetic construct
  misc_feature 1..23: note = CXCR4 gRNA target site sequence
  source 1..23: mol_type = other DNA
ctcctggaaatcatcaagcaagg

SEQ ID NO: 237 - DNA, 23 bp, synthetic construct
  misc_feature 1..23: note = CXCR4 gRNA target site sequence
  source 1..23: mol_type = other DNA
catcgactccttcatcctcctgg

SEQ ID NO: 238 - DNA, 23 bp, synthetic construct
  misc_feature 1..23: note = CXCR4 gRNA target site sequence
  source 1..23: mol_type = other DNA
gttggctgccttactacattggg

SEQ ID NO: 239 - DNA, 23 bp, synthetic construct
  misc_feature 1..23: note = CXCR4 gRNA target site sequence
  source 1..23: mol_type = other DNA
tgttggctgccttactacattgg

SEQ ID NO: 240 - DNA, 23 bp, synthetic construct
  misc_feature 1..23: note = CXCR4 gRNA target site sequence
  source 1..23: mol_type = other DNA
tcctggctttcttcgcctgttgg

SEQ ID NO: 241 - DNA, 23 bp, synthetic construct
  misc_feature 1..23: note = CXCR4 gRNA target site sequence
  source 1..23: mol_type = other DNA
gaccacagtcatcctcatcctgg

SEQ ID NO: 242 - DNA, 23 bp, synthetic construct
  misc_feature 1..23: note = CXCR4 gRNA target site sequence
  source 1..23: mol_type = other DNA
caagggccaccagaagcgcaagg

SEQ ID NO: 243 - DNA, 23 bp, synthetic construct
  misc_feature 1..23: note = CXCR4 gRNA target site sequence
  source 1..23: mol_type = other DNA
tccaagctgtcacactccaaggg

SEQ ID NO: 244 - DNA, 23 bp, synthetic construct
  misc_feature 1..23: note = CXCR4 gRNA target site sequence
  source 1..23: mol_type = other DNA
ctccaagctgtcacactccaagg

SEQ ID NO: 245 - DNA, 23 bp, synthetic construct
  misc_feature 1..23: note = CXCR4 gRNA target site sequence
  source 1..23: mol_type = other DNA
atggttggccttatcctgcctgg

SEQ ID NO: 246 - DNA, 23 bp, synthetic construct
  misc_feature 1..23: note = CXCR4 gRNA target site sequence
  source 1..23: mol_type = other DNA
cagtttcagcacatcatggttgg

SEQ ID NO: 247 - DNA, 23 bp, synthetic construct
  misc_feature 1..23: note = CXCR4 gRNA target site sequence
  source 1..23: mol_type = other DNA
gttccagtttcagcacatcatgg

SEQ ID NO: 248 - DNA, 23 bp, synthetic construct
  misc_feature 1..23: note = CXCR4 gRNA target site sequence
  source 1..23: mol_type = other DNA
ctaccccaatgacttgtgggtgg

SEQ ID NO: 249 - DNA, 23 bp, synthetic construct
  misc_feature 1..23: note = CXCR4 gRNA target site sequence
  source 1..23: mol_type = other DNA
cttctaccccaatgacttgtggg

SEQ ID NO: 250 - DNA, 23 bp, synthetic construct
  misc_feature 1..23: note = CXCR4 gRNA target site sequence
  source 1..23: mol_type = other DNA
gcttctaccccaatgacttgtgg

SEQ ID NO: 251 - DNA, 23 bp, synthetic construct
  misc_feature 1..23: note = CXCR4 gRNA target site sequence
  source 1..23: mol_type = other DNA
catctttgccaacgtcagtgagg

SEQ ID NO: 252 - DNA, 23 bp, synthetic construct
  misc_feature 1..23: note = CXCR4 gRNA target site sequence
  source 1..23: mol_type = other DNA
aggtggtctatgttggcgtctgg

SEQ ID NO: 253 - DNA, 23 bp, synthetic construct
  misc_feature 1..23: note = CXCR4 gRNA target site sequence
  source 1..23: mol_type = other DNA
gctgaaaaggtggtctatgttgg

SEQ ID NO: 254 - DNA, 23 bp, synthetic construct
  misc_feature 1..23: note = CXCR4 gRNA target site sequence
  source 1..23: mol_type = other DNA
gaagctgttggctgaaaaggtgg

SEQ ID NO: 255 - DNA, 23 bp, synthetic construct
  misc_feature 1..23: note = CXCR4 gRNA target site sequence
  source 1..23: mol_type = other DNA
aaggaagctgttggctgaaaagg

SEQ ID NO: 256 - DNA, 23 bp, synthetic construct
  misc_feature 1..23: note = CXCR4 gRNA target site sequence
  source 1..23: mol_type = other DNA
tcagaggccaaggaagctgttgg

SEQ ID NO: 257 - DNA, 23 bp, synthetic construct
  misc_feature 1..23: note = CXCR4 gRNA target site sequence
  source 1..23: mol_type = other DNA
ccaccaacagtcagaggccaagg

SEQ ID NO: 258 - DNA, 23 bp, synthetic construct
  misc_feature 1..23: note = CXCR4 gRNA target site sequence
  source 1..23: mol_type = other DNA
tccacgccaccaacagtcagagg

SEQ ID NO: 259 - DNA, 23 bp, synthetic construct
  misc_feature 1..23: note = CXCR4 gRNA target site sequence
  source 1..23: mol_type = other DNA
catcagtctggaccgctacctgg

SEQ ID NO: 260 - DNA, 23 bp, synthetic construct
  misc_feature 1..23: note = CXCR4 gRNA target site sequence
  source 1..23: mol_type = other DNA
catcctggccttcatcagtctgg

SEQ ID NO: 261 - DNA, 23 bp, synthetic construct
  misc_feature 1..23: note = CXCR4 gRNA target site sequence
  source 1..23: mol_type = other DNA
ctacagcagtgtcctcatcctgg

SEQ ID NO: 262 - DNA, 23 bp, synthetic construct
  misc_feature 1..23: note = CXCR4 gRNA target site sequence
  source 1..23: mol_type = other DNA
ctttgggaacttcctatgcaagg

SEQ ID NO: 263 - DNA, 23 bp, synthetic construct
  misc_feature 1..23: note = CXCR4 gRNA target site sequence
  source 1..23: mol_type = other DNA
ccgtggcaaactggtactttggg

SEQ ID NO: 264 - DNA, 23 bp, synthetic construct
  misc_feature 1..23: note = CXCR4 gRNA target site sequence
  source 1..23: mol_type = other DNA
gccgtggcaaactggtactttgg

SEQ ID NO: 265 - DNA, 23 bp, synthetic construct
  misc_feature 1..23: note = CXCR4 gRNA target site sequence
  source 1..23: mol_type = other DNA
cagttgatgccgtggcaaactgg

SEQ ID NO: 266 - DNA, 23 bp, synthetic construct
  misc_feature 1..23: note = CXCR4 gRNA target site sequence
  source 1..23: mol_type = other DNA
cttctgggcagttgatgccgtgg

SEQ ID NO: 267 - DNA, 23 bp, synthetic construct
  misc_feature 1..23: note = CXCR4 gRNA target site sequence
  source 1..23: mol_type = other DNA
tgtcatcacgcttcccttctggg

SEQ ID NO: 268 - DNA, 23 bp, synthetic construct
  misc_feature 1..23: note = CXCR4 gRNA target site sequence
  source 1..23: mol_type = other DNA
ttgtcatcacgcttcccttctgg

SEQ ID NO: 269 - DNA, 23 bp, synthetic construct
  misc_feature 1..23: note = CXCR4 gRNA target site sequence
  source 1..23: mol_type = other DNA
gtacaggctgcacctgtcagtgg

SEQ ID NO: 270 - DNA, 23 bp, synthetic construct
  misc_feature 1..23: note = CXCR4 gRNA target site sequence
  source 1..23: mol_type = other DNA
gaagcatgacggacaagtacagg

SEQ ID NO: 271 - DNA, 23 bp, synthetic construct
  misc_feature 1..23: note = CXCR4 gRNA target site sequence
  source 1..23: mol_type = other DNA
gaagaaactgagaagcatgacgg

SEQ ID NO: 272 - DNA, 23 bp, synthetic construct
  misc_feature 1..23: note = CXCR4 gRNA target site sequence
  source 1..23: mol_type = other DNA
ggattggtcatcctggtcatggg

SEQ ID NO: 273 - DNA, 23 bp, synthetic construct
  misc_feature 1..23: note = CXCR4 gRNA target site sequence
  source 1..23: mol_type = other DNA
tggattggtcatcctggtcatgg

SEQ ID NO: 274 - DNA, 23 bp, synthetic construct
  misc_feature 1..23: note = CXCR4 gRNA target site sequence
  source 1..23: mol_type = other DNA
gggcaatggattggtcatcctgg

SEQ ID NO: 275 - DNA, 23 bp, synthetic construct
  misc_feature 1..23: note = CXCR4 gRNA target site sequence
  source 1..23: mol_type = other DNA
tggcattgtgggcaatggattgg

SEQ ID NO: 276 - DNA, 23 bp, synthetic construct
  misc_feature 1..23: note = CXCR4 gRNA target site sequence
  source 1..23: mol_type = other DNA
ttaactggcattgtgggcaatgg

SEQ ID NO: 277 - DNA, 23 bp, synthetic construct
  misc_feature 1..23: note = CXCR4 gRNA target site sequence
  source 1..23: mol_type = other DNA
atcttcttaactggcattgtggg

SEQ ID NO: 278 - DNA, 23 bp, synthetic construct
  misc_feature 1..23: note = CXCR4 gRNA target site sequence
  source 1..23: mol_type = other DNA
catcttcttaactggcattgtgg

SEQ ID NO: 279 - DNA, 23 bp, synthetic construct
  misc_feature 1..23: note = CXCR4 gRNA target site sequence
  source 1..23: mol_type = other DNA
tactccatcatcttcttaactgg

SEQ ID NO: 280 - DNA, 23 bp, synthetic construct
  misc_feature 1..23: note = CXCR4 gRNA target site sequence
  source 1..23: mol_type = other DNA
aggggactatgactccatgaagg

SEQ ID NO: 281 - DNA, 23 bp, synthetic construct
  misc_feature 1..23: note = CXCR4 gRNA target site sequence
  source 1..23: mol_type = other DNA
caccgaggaaatgggctcagggg

SEQ ID NO: 282 - DNA, 23 bp, synthetic construct
  misc_feature 1..23: note = CXCR4 gRNA target site sequence
  source 1..23: mol_type = other DNA
acaccgaggaaatgggctcaggg

SEQ ID NO: 283 - DNA, 23 bp, synthetic construct
  misc_feature 1..23: note = CXCR4 gRNA target site sequence
  source 1..23: mol_type = other DNA
tacaccgaggaaatgggctcagg

SEQ ID NO: 284 - DNA, 23 bp, synthetic construct
  misc_feature 1..23: note = CXCR4 gRNA target site sequence
  source 1..23: mol_type = other DNA
gataactacaccgaggaaatggg

SEQ ID NO: 285 - DNA, 23 bp, synthetic construct
  misc_feature 1..23: note = CXCR4 gRNA target site sequence
  source 1..23: mol_type = other DNA
agataactacaccgaggaaatgg

SEQ ID NO: 286 - DNA, 23 bp, synthetic construct
  misc_feature 1..23: note = CXCR4 gRNA target site sequence
  source 1..23: mol_type = other DNA
cacttcagataactacaccgagg

SEQ ID NO: 287 - DNA, 28 bp, synthetic construct
  misc_feature 1..28: note = CXCR4 gRNA target site sequence
  source 1..28: mol_type = other DNA
gatggggttcagacaacagtggaagaaa

SEQ ID NO: 288 - DNA, 28 bp, synthetic construct
  misc_feature 1..28: note = CXCR4 gRNA target site sequence
  source 1..28: mol_type = other DNA
gtagtaaggcagccaacaggcgaagaaa

SEQ ID NO: 289 - DNA, 28 bp, synthetic construct
  misc_feature 1..28: note = CXCR4 gRNA target site sequence
  source 1..28: mol_type = other DNA
aaccacccacaagtcattggggtagaag

SEQ ID NO: 290 - DNA, 28 bp, synthetic construct
  misc_feature 1..28: note = CXCR4 gRNA target site sequence
  source 1..28: mol_type = other DNA
gtttgccacggcatcaactgcccagaag

SEQ ID NO: 291 - DNA, 28 bp, synthetic construct
  misc_feature 1..28: note = CXCR4 gRNA target site sequence
  source 1..28: mol_type = other DNA
tccattgcccacaatgccagttaagaag

SEQ ID NO: 292 - DNA, 28 bp, synthetic construct
  misc_feature 1..28: note = CXCR4 gRNA target site sequence
  source 1..28: mol_type = other DNA
catcaagcaagggtgtgagtttgagaac

SEQ ID NO: 293 - DNA, 28 bp, synthetic construct
  misc_feature 1..28: note = CXCR4 gRNA target site sequence
  source 1..28: mol_type = other DNA
gctgtcacactccaagggccaccagaag

SEQ ID NO: 294 - DNA, 28 bp, synthetic construct
  misc_feature 1..28: note = CXCR4 gRNA target site sequence
  source 1..28: mol_type = other DNA
tcatgggttaccagaagaaactgagaag

SEQ ID NO: 295 - DNA, 28 bp, synthetic construct
  misc_feature 1..28: note = CXCR4 gRNA target site sequence
  source 1..28: mol_type = other DNA
catcctggtcatgggttaccagaagaaa

SEQ ID NO: 296 - DNA, 28 bp, synthetic construct
  misc_feature 1..28: note = CXCR4 gRNA target site sequence
  source 1..28: mol_type = other DNA
ggtcatcctggtcatgggttaccagaag

SEQ ID NO: 297 - DNA, 28 bp, synthetic construct
  misc_feature 1..28: note = CXCR4 gRNA target site sequence
  source 1..28: mol_type = other DNA
atgaaggaaccctgtttccgtgaagaaa

SEQ ID NO: 298 - DNA, 20 bp, synthetic construct
  misc_feature 1..20: note = gRNA
  source 1..20: mol_type = other DNA
gtcttgctcgagatgtgatg

SEQ ID NO: 299 - DNA, 20 bp, synthetic construct
  misc_feature 1..20: note = gRNA
  source 1..20: mol_type = other DNA
taaattctttgctgacctgc

SEQ ID NO: 300 - DNA, 20 bp, synthetic construct
  misc_feature 1..20: note = gRNA
  source 1..20: mol_type = other DNA
tagatccattcctatgactg

SEQ ID NO: 301 - DNA, 20 bp, synthetic construct
  misc_feature 1..20: note = gRNA
  source 1..20: mol_type = other DNA
cttcagtctgataaaatcta

SEQ ID NO: 302 - DNA, 20 bp, synthetic construct
  misc_feature 1..20: note = gRNA
  source 1..20: mol_type = other DNA
tttgatgtaatccagcaggt

SEQ ID NO: 303 - DNA, 20 bp, synthetic construct
  misc_feature 1..20: note = gRNA
  source 1..20: mol_type = other DNA
cacagagggctacaatgtga

SEQ ID NO: 304 - DNA, 23 bp, synthetic construct
  misc_feature 1..23: note = Target site sequence with NGG
  source 1..23: mol_type = other DNA
gtagagcggaggcaggaggcggg

SEQ ID NO: 305 - DNA, 23 bp, synthetic construct
  misc_feature 1..23: note = Target site sequence with NGG
  source 1..23: mol_type = other DNA
gtgagtagagcggaggcaggagg

SEQ ID NO: 306 - DNA, 23 bp, synthetic construct
  misc_feature 1..23: note = Target site sequence with NGG
  source 1..23: mol_type = other DNA
ggtgttcatctttggttttgtgg

SEQ ID NO: 307 - DNA, 23 bp, synthetic construct
  misc_feature 1..23: note = Target site sequence with NGG
  source 1..23: mol_type = other DNA
gtgttcatctttggttttgtggg

SEQ ID NO: 308 - DNA, 23 bp, synthetic construct
  misc_feature 1..23: note = Target site sequence with NGG
  source 1..23: mol_type = other DNA
ggacagtaagaaggaaaaacagg

SEQ ID NO: 309 - DNA, 23 bp, synthetic construct
  misc_feature 1..23: note = Target site sequence with NGG
  source 1..23: mol_type = other DNA
gctgccgcccagtgggactttgg

SEQ ID NO: 310 - DNA, 23 bp, synthetic construct
  misc_feature 1..23: note = Target site sequence with NGG
  source 1..23: mol_type = other DNA
gcagcatagtgagcccagaaggg

SEQ ID NO: 311 - DNA, 23 bp, synthetic construct
  misc_feature 1..23: note = Target site sequence with NGG
  source 1..23: mol_type = other DNA
ggcagcatagtgagcccagaagg

SEQ ID NO: 312 - DNA, 23 bp, synthetic construct
  misc_feature 1..23: note = Target site sequence with NGG
  source 1..23: mol_type = other DNA
ggtacctatcgattgtcaggagg

SEQ ID NO: 313 - DNA, 23 bp, synthetic construct
  misc_feature 1..23: note = Target site sequence with NGG
  source 1..23: mol_type = other DNA
gtttgctttaaaagccaggacgg

SEQ ID NO: 314 - DNA, 23 bp, synthetic construct
  misc_feature 1..23: note = Target site sequence with NGG
  source 1..23: mol_type = other DNA
ggtgacaagtgtgatcacttggg

SEQ ID NO: 315 - DNA, 23 bp, synthetic construct
  misc_feature 1..23: note = Target site sequence with NGG
  source 1..23: mol_type = other DNA
gacaagtgtgatcacttgggtgg

SEQ ID NO: 316 - DNA, 23 bp, synthetic construct
  misc_feature 1..23: note = Target site sequence with NGG
  source 1..23: mol_type = other DNA
gctgtgtttgcgtctctcccagg

SEQ ID NO: 317 - DNA, 23 bp, synthetic construct
  misc_feature 1..23: note = Target site sequence with NGG
  source 1..23: mol_type = other DNA
gatctggtaaagatgattcctgg

SEQ ID NO: 318 - DNA, 23 bp, synthetic construct
  misc_feature 1..23: note = Target site sequence with NGG
  source 1..23: mol_type = other DNA
gtatggaaaatgagagctgcagg

SEQ ID NO: 319 - DNA, 23 bp, synthetic construct
  misc_feature 1..23: note = Target site sequence with NGG
  source 1..23: mol_type = other DNA
gacattaaagatagtcatcttgg

SEQ ID NO: 320 - DNA, 23 bp, synthetic construct
  misc_feature 1..23: note = Target site sequence with NGG
  source 1..23: mol_type = other DNA
ggtcctgccgctgcttgtcatgg

SEQ ID NO: 321 - DNA, 23 bp, synthetic construct
  misc_feature 1..23: note = Target site sequence with NGG
  source 1..23: mol_type = other DNA
gtcatggtcatctgctactcggg

SEQ ID NO: 322 - DNA, 23 bp, synthetic construct
  misc_feature 1..23: note = Target site sequence with NGG
  source 1..23: mol_type = other DNA
gaatcctaaaaactctgcttcgg

SEQ ID NO: 323 - DNA, 23 bp, synthetic construct
  misc_feature 1..23: note = Target site sequence with NGG
  source 1..23: mol_type = other DNA
ggtgtcgaaatgagaagaagagg

SEQ ID NO: 324 - DNA, 23 bp, synthetic construct
  misc_feature 1..23: note = Target site sequence with NGG
  source 1..23: mol_type = other DNA
gacaccgaagcagagtttttagg

SEQ ID NO: 325 - DNA, 23 bp, synthetic construct
  misc_feature 1..23: note = Target site sequence with NGG
  source 1..23: mol_type = other DNA
gaaatgagaagaagaggcacagg

SEQ ID NO: 326 - DNA, 23 bp, synthetic construct
  misc_feature 1..23: note = Target site sequence with NGG
  source 1..23: mol_type = other DNA
gattgtttattttctcttctggg

SEQ ID NO: 327 - DNA, 23 bp, synthetic construct
  misc_feature 1..23: note = Target site sequence with NGG
  source 1..23: mol_type = other DNA
gagaaaataaacaatcatgatgg

SEQ ID NO: 328 - DNA, 23 bp, synthetic construct
  misc_feature 1..23: note = Target site sequence with NGG
  source 1..23: mol_type = other DNA
gcttttggaagaagactaagagg

SEQ ID NO: 329 - DNA, 23 bp, synthetic construct
  misc_feature 1..23: note = Target site sequence with NGG
  source 1..23: mol_type = other DNA
gtaaactgagcttgctcgctcgg

SEQ ID NO: 330 - DNA, 23 bp, synthetic construct
  misc_feature 1..23: note = Target site sequence with NGG
  source 1..23: mol_type = other DNA
ggggagcaggaaatatctgtggg

SEQ ID NO: 331 - DNA, 23 bp, synthetic construct
  misc_feature 1..23: note = Target site sequence with NGG
  source 1..23: mol_type = other DNA
acaatgtgtcaactcttgacagg

SEQ ID NO: 332 - DNA, 23 bp, synthetic construct
  misc_feature 1..23: note = Target site sequence with NGG
  source 1..23: mol_type = other DNA
tcactatgctgccgcccagtggg

SEQ ID NO: 333 - DNA, 23 bp, synthetic construct
  misc_feature 1..23: note = Target site sequence with NGG
  source 1..23: mol_type = other DNA
ggtacctatcgattgtcaggagg

SEQ ID NO: 334 - protein, 1368 aa, unidentified [sequence omitted]

SEQ ID NO: 335 - DNA, 47 bp, synthetic construct
  misc_feature 1..47: note = target sequence
  source 1..47: mol_type = other DNA
tcccttcctgcctcatttcaggtgaatacatcaagacctggaggcca

SEQ ID NO: 336 - DNA, 47 bp, synthetic construct; identical to SEQ ID NO: 335
  misc_feature 1..47: note = target sequence
  source 1..47: mol_type = other DNA

SEQ ID NO: 337 - DNA, 47 bp, synthetic construct
  misc_feature 1..47: note = target sequence
  source 1..47: mol_type = other DNA
tgctggctcggctgccctgaggttgctcaatcaagcacaggtttcaa

SEQ ID NO: 338 - DNA, 47 bp, synthetic construct; identical to SEQ ID NO: 337
  misc_feature 1..47: note = target sequence
  source 1..47: mol_type = other DNA

SEQ ID NO: 339 - DNA, 47 bp, synthetic construct
  misc_feature 1..47: note = target sequence
  source 1..47: mol_type = other DNA
taacagcgatgctgaccccctgtgcctctaccacttctatgaccaga

SEQ ID NO: 340 - DNA, 47 bp, synthetic construct
  misc_feature 1..47: note = target sequence
  source 1..47: mol_type = other DNA
cgatgctgaccccctgtgcctctaccacttctatgaccagatggacc

SEQ ID NO: 341 - DNA, 49 bp, synthetic construct
  misc_feature 1..49: note = target sequence
  source 1..49: mol_type = other DNA
tggtccttgctgtgttctctgcggtgcttggctccctgcagtttgggta

SEQ ID NO: 342 - DNA, 49 bp, synthetic construct; identical to SEQ ID NO: 341
  misc_feature 1..49: note = target sequence
  source 1..49: mol_type = other DNA

SEQ ID NO: 343 - DNA, 47 bp, synthetic construct
  misc_feature 1..47: note = target sequence
  source 1..47: mol_type = other DNA
tgggcgacagatgcgaaagaaacgagttccagtgccaagacgggaaa

SEQ ID NO: 344 - DNA, 47 bp, synthetic construct
  misc_feature 1..47: note = target sequence
  source 1..47: mol_type = other DNA
gaaacgagttccagtgccaagacgggaaatgcatctcctacaagtgg

SEQ ID NO: 345 - DNA, 48 bp, synthetic construct
  misc_feature 1..48: note = target sequence
  source 1..48: mol_type = other DNA
tcagagaggacactgcagttgtccgtgctagtagccttcgcttctgga

SEQ ID NO: 346 - DNA, 48 bp, synthetic construct; identical to SEQ ID NO: 345
  misc_feature 1..48: note = target sequence
  source 1..48: mol_type = other DNA

SEQ ID NO: 347 - DNA, 47 bp, synthetic construct
  misc_feature 1..47: note = target sequence
  source 1..47: mol_type = other DNA
tgatgatctcagaggctcagtatccttgtcctgggttggagatagca

SEQ ID NO: 348 - DNA, 47 bp, synthetic construct; identical to SEQ ID NO: 347
  misc_feature 1..47: note = target sequence
  source 1..47: mol_type = other DNA

SEQ ID NO: 349 - DNA, 49 bp, synthetic construct
  misc_feature 1..49: note = target sequence
  source 1..49: mol_type = other DNA
tggtaattatgacttttggacagtccaagctatatcgaaggtgagatca

SEQ ID NO: 350 - DNA, 49 bp, synthetic construct; identical to SEQ ID NO: 349
  misc_feature 1..49: note = target sequence
  source 1..49: mol_type = other DNA

SEQ ID NO: 351 - DNA, 47 bp, synthetic construct; identical to SEQ ID NO: 335
  misc_feature 1..47: note = target sequence
  source 1..47: mol_type = other DNA

SEQ ID NO: 352 - DNA, 47 bp, synthetic construct; identical to SEQ ID NO: 335
  misc_feature 1..47: note = target sequence
  source 1..47: mol_type = other DNA

SEQ ID NO: 353 - DNA, 47 bp, synthetic construct
  misc_feature 1..47: note = target sequence
  source 1..47: mol_type = other DNA
ctatgccctgcctcatttcaggtgaagatgaaatccctggagcttgg